European Patent Application EP 4 741 497 A1, published May 13, 2026. Title: 一种新型CRISPR酶和系统及应用. Applicant: 山东舜丰生物科技有限公司. Application CN. The sequence listing filed with the application follows.

SEQUENCE LISTING (31 sequences)

SEQ ID NO: 1 - protein, 460 aa, unidentified
  REGION 1..460: note = Cas-sf6728
MADESTKPKTHIRTLKLKLKVVGDDPKTSWKRLRQTSNDTWRAANWIAAGQFMNDQLVRRLYARLKVDSKDPAAVQKVEDDFKAVFGTKRQATTERDIKQQFPDLPPCVTNTLNQFVVASYTKEKPDMLAGNRSLRTYRKGLPIPTSRASVDFSAQDGRHIVSWKVQRGEQIQFEVFYGRDKAGNERTIGLIIATERDYGAPSIQLNEKGLFLLLPVKEPAQDATLDPKRVVGVDLGLAVPAYAAVSDGPARRPMGSAEDFLKTRLQMQSRRRRLQRSLVAVHGGNGRQRKMKAMDRLSEKERHFARTYNHMISRRLVDFALQVGAGQINMELLEGFGRDEQQAFVLRNWSFFELQQLIGEKAARVGIKVRHVDPYHTSQICSECGNWAQGQRDGRDFVCQNCGLKLDADYNAAVNISRSTKYVQRKEQCRAYIERQTTTTESDDIEKSETDSAGPTAEG

SEQ ID NO: 2 - DNA, 1383 bp, unidentified
  source 1..1383: mol_type = other DNA
  misc_feature 1..1383: note = Cas-sf6728
atggccgatgaaagcaccaaaccgaaaacccatattcgcaccctgaaactgaaactgaaggttgtgggtgatgatccgaaaaccagctggaaacgtctgcgtcagaccagcaatgatacctggcgtgcagcaaattggattgccgccggtcagtttatgaatgatcagctggtgcgtcgtctgtatgcacgtctgaaagttgatagcaaagatccggccgccgtgcagaaagttgaagatgattttaaagccgttttcggtaccaaacgccaggcaaccaccgaacgtgatattaaacagcagtttccggatctgccgccgtgtgtgaccaataccctgaatcagtttgtggttgcaagttataccaaagaaaaaccggatatgctggcaggcaatcgcagcctgcgtacctatcgcaaaggtctgccgattccgaccagccgcgccagtgtggattttagcgcacaggatggtcgtcatattgttagctggaaagttcagcgcggcgaacagattcagtttgaagttttttatggccgtgataaagcaggcaatgaacgcaccattggtctgattattgcaaccgaacgtgactatggtgcacctagtattcagctgaatgaaaaaggcctgtttctgctgctgccggttaaagaaccggcccaggatgcaaccctggaccctaaacgcgtggttggtgttgatctgggtctggccgtgccggcatatgccgccgtgagcgatggcccggcccgtcgtcctatgggtagtgcagaagattttctgaaaacccgtctgcagatgcagagccgccgccgccgtctgcagcgtagtctggttgccgtgcatggtggcaatggccgtcagcgtaaaatgaaagccatggatcgtctgagtgaaaaagaacgtcattttgcccgcacctataatcatatgattagtcgccgcctggtggattttgccctgcaggttggtgccggtcagattaatatggaactgctggaaggctttggccgtgatgaacagcaggcctttgttctgcgcaattggagcttttttgaactgcagcagctgattggtgaaaaagcagcacgtgtgggtattaaagttcgtcatgtggacccttatcataccagccagatttgcagtgaatgtggcaattgggcacagggccagcgcgatggccgtgattttgtgtgccagaattgcggtctgaaactggatgcagattataatgcagcagtgaatattagccgtagcaccaaatatgtgcagcgtaaagaacagtgtcgtgcctatattgaacgccagaccaccaccaccgaaagcgatgatattgaaaaaagtgaaaccgatagcgcaggcccgaccgcagaaggctaa

SEQ ID NO: 3 - RNA, 29 nt, unidentified
  source 1..29: mol_type = other RNA
  misc_feature 1..29: note = Cas-sf6728
aacgagcccacgcgtgccgggatgggtcg

SEQ ID NO: 4 - RNA, 200 nt, unidentified
  source 1..200: mol_type = other RNA
  misc_feature 1..200: note = Cas-sf6728
tcaaccaaatatgtccaacgaaaggagcaatgccgggcctacatcgagcgacaaaccacaacaaccgaatccgacgatatcgagaagtcggaaactgattcggctgggcccacagccgaagggtgagggctaagcgccactcaccaaccccgcatgcgcaatatattgcgacttggctcgtcccacagcacaacatggca

SEQ ID NO: 5 - RNA, 233 nt, unidentified
  source 1..233: mol_type = other RNA
  misc_feature 1..233: note = wild type
tcaaccaaatatgtccaacgaaaggagcaatgccgggcctacatcgagcgacaaaccacaacaaccgaatccgacgatatcgagaagtcggaaactgattcggctgggcccacagccgaagggtgagggctaagcgccactcaccaaccccgcatgcgcaatatattgcgacttggctcgtcccacagcacaacatggcagaaaaacgagcccacgcgtgccgggatgggtcg

SEQ ID NO: 6 - RNA, 221 nt, unidentified
  source 1..221: mol_type = other RNA
  misc_feature 1..221: note = A1
gtccaacgaaaggagcaatgccgggcctacatcgagcgacaaaccacaacaaccgaatccgacgatatcgagaagtcggaaactgattcggctgggcccacagccgaagggtgagggctaagcgccactcaccaaccccgcatgcgcaatatattgcgacttggctcgtcccacagcacaacatggcagaaaaacgagcccacgcgtgccgggatgggtcg

SEQ ID NO: 7 - RNA, 207 nt, unidentified
  source 1..207: mol_type = other RNA
  misc_feature 1..207: note = A2
gcaatgccgggcctacatcgagcgacaaaccacaacaaccgaatccgacgatatcgagaagtcggaaactgattcggctgggcccacagccgaagggtgagggctaagcgccactcaccaaccccgcatgcgcaatatattgcgacttggctcgtcccacagcacaacatggcagaaaaacgagcccacgcgtgccgggatgggtcg

SEQ ID NO: 8 - RNA, 204 nt, unidentified
  source 1..204: mol_type = other RNA
  misc_feature 1..204: note = A3
tcaaccaaatatgcaatgccgggcctacatcgagcgacaaaccacaacaaccgaatccgacgatatcgagaagtcggaaactgattcggctgggcccacagccgaagggtgagggctaagcgccactcaccaaccccgcatgcttggctcgtcccacagcacaacatggcagaaaaacgagcccacgcgtgccgggatgggtcg

SEQ ID NO: 9 - RNA, 233 nt, unidentified
  source 1..233: mol_type = other RNA
  misc_feature 1..233: note = A4
tcaaccaaatatgtccaacgaaaggagccatgccgggcctacatcgagcgacaaaccacaacaaccgaatccgacgatatcgagaagtcggaaactgattcggctgggcccacagccgaagggtgagggctaagcgccactcaccaaccccgcaggcgcaatatattgcgacttggctcgtcccacagcacaacatggcagaaaaacgagcccacgcgtgccgggatgggtcg

SEQ ID NO: 10 - RNA, 233 nt, unidentified
  source 1..233: mol_type = other RNA
  misc_feature 1..233: note = A5
tcaaccaaatatgtccaacgaaaggagcaacgccgggcctacatcgagcgacaaaccacaacaaccgaatccgacgatatcgagaagtcggaaactgattcggctgggcccacagccgaagggtgagggctaagcgccactcaccaaccccgcgtgcgcaatatattgcgacttggctcgtcccacagcacaacatggcagaaaaacgagcccacgcgtgccgggatgggtcg

SEQ ID NO: 11 - RNA, 234 nt, unidentified
  source 1..234: mol_type = other RNA
  misc_feature 1..234: note = A6
tcaaccaaatatgtccaacgaaaggagcaatgccgggcctacatcgagcgacaaaccacaacaaccgaatccgacgatatcgagaagtcggaaactgattcggctgggcccacagccgaagggtgagggctaagcgccactcaccaaccccgcattgcgcaatatattgcgacttggctcgtcccacagcacaacatggcagaaaaacgagcccacgcgtgccgggatgggtcg

SEQ ID NO: 12 - RNA, 233 nt, unidentified
  source 1..233: mol_type = other RNA
  misc_feature 1..233: note = A7
tcaaccaaatatgtccaacgaaaggagccacgccgggcctacatcgagcgacaaaccacaacaaccgaatccgacgatatcgagaagtcggaaactgattcggctgggcccacagccgaagggtgagggctaagcgccactcaccaaccccgcgggcgcaatatattgcgacttggctcgtcccacagcacaacatggcagaaaaacgagcccacgcgtgccgggatgggtcg

SEQ ID NO: 13 - RNA, 233 nt, unidentified
  source 1..233: mol_type = other RNA
  misc_feature 1..233: note = A8
tcaaccaaatatgtccaacgaaaggagcaatgccgggcctacatcgagcgacaaaccacaacaaccgaatccgccgatatcgagaaggcggaaactgattcggctgggcccacagccgaagggtgagggctaagcgccactcaccaaccccgcatgcgcaatatattgcgacttggctcgtcccacagcacaacatggcagaaaaacgagcccacgcgtgccgggatgggtcg

SEQ ID NO: 14 - RNA, 233 nt, unidentified
  source 1..233: mol_type = other RNA
  misc_feature 1..233: note = A9
tcaaccaaatatgtccaacgaaaggagcaatgccgggcctacatcgagcgacaaaccacaacaaccgaatccgacgatatcgagaagtcggaaactgatccggctgggcccacagccggagggtgagggctaagcgccactcaccaaccccgcatgcgcaatatattgcgacttggctcgtcccacagcacaacatggcagaaaaacgagcccacgcgtgccgggatgggtcg

SEQ ID NO: 15 - RNA, 233 nt, unidentified
  source 1..233: mol_type = other RNA
  misc_feature 1..233: note = A10
tcaaccaaatatgtccaacgaaaggagcaatgccgggcctacatcgagcgacaaaccacaacaaccgaatccgacgatatcgagaagtcggaaactgattcggccgggcccacggccgaagggtgagggctaagcgccactcaccaaccccgcatgcgcaatatattgcgacttggctcgtcccacagcacaacatggcagaaaaacgagcccacgcgtgccgggatgggtcg

SEQ ID NO: 16 - RNA, 233 nt, unidentified
  source 1..233: mol_type = other RNA
  misc_feature 1..233: note = A11
tcaaccaaatatgtccaacgaaaggagcaatgccgggcctacatcgagcgacaaaccacaacaaccgaatccgacgatatcgagaagtcggaaactgatccggccgggcccacggccggagggtgagggctaagcgccactcaccaaccccgcatgcgcaatatattgcgacttggctcgtcccacagcacaacatggcagaaaaacgagcccacgcgtgccgggatgggtcg

SEQ ID NO: 17 - RNA, 233 nt, unidentified
  source 1..233: mol_type = other RNA
  misc_feature 1..233: note = A12
tcaaccaaatatgtccaacgaaaggagcaatgccgggcctacatcgagcgacaaaccacaacaaccgaatccgacgatatcgagaagtcggaaactgattcggctgggcccacagccgaagggggagggctaagcgccactccccaaccccgcatgcgcaatatattgcgacttggctcgtcccacagcacaacatggcagaaaaacgagcccacgcgtgccgggatgggtcg

SEQ ID NO: 18 - RNA, 233 nt, unidentified
  source 1..233: mol_type = other RNA
  misc_feature 1..233: note = A13
tcaaccaaatatgtccaacgaaaggagcaatgccgggcctacatcgagcgacaaaccacaacaaccgaatccgacgatatcgagaagtcggaaactgattcggctgggcccacagccgaagggtgggggctaagcgccacccaccaaccccgcatgcgcaatatattgcgacttggctcgtcccacagcacaacatggcagaaaaacgagcccacgcgtgccgggatgggtcg

SEQ ID NO: 19 - RNA, 234 nt, unidentified
  source 1..234: mol_type = other RNA
  misc_feature 1..234: note = A14
tcaaccaaatatgtccaacgaaaggagcaatgccgggcctacatcgagcgacaaaccacaacaaccgaatccgacgatatcgagaagtcggaaactgattcggctgggcccacagccgaagggtgagtggctaagcgccactcaccaaccccgcatgcgcaatatattgcgacttggctcgtcccacagcacaacatggcagaaaaacgagcccacgcgtgccgggatgggtcg

SEQ ID NO: 20 - RNA, 233 nt, unidentified
  source 1..233: mol_type = other RNA
  misc_feature 1..233: note = A15
tcaaccaaatatgtccaacgaaaggagcaatgccgggcctacatcgagcgacaaaccacaacaaccgaatccgacgatatcgagaagtcggaaactgattcggctgggcccacagccgaagggggggggctaagcgccaccccccaaccccgcatgcgcaatatattgcgacttggctcgtcccacagcacaacatggcagaaaaacgagcccacgcgtgccgggatgggtcg

SEQ ID NO: 21 - RNA, 229 nt, unidentified
  source 1..229: mol_type = other RNA
  misc_feature 1..229: note = A16
tcaaccaaatatgtccaacgaaaggagcaatgccgggcctacatcgagcgacaaaccacaacaaccgaatccgacgatatcgagaagtcggaaactgattcggctgggcccacagccgaagggtgagggctaagcgccactcaccaaccccgcatgcgcaatatattgcgacttggctcgtcccacagcacaacatgaaaaacgagcccacgcgtgccgggatgggtcg

SEQ ID NO: 22 - RNA, 224 nt, unidentified
  source 1..224: mol_type = other RNA
  misc_feature 1..224: note = A17
tcaaccaaatatgtccaacgaaaggagcaatgccgggcctacatcgagcgacaaaccacaacaaccgaatccgacgatatcgagaagtcggaaactgattcggctgggcccacagccgaagggtgagggctaagcgccactcaccaaccccgcatgcgcaatatattgcgacttggctcgtcccacagcacgaaaaacgagcccacgcgtgccgggatgggtcg

SEQ ID NO: 23 - RNA, 228 nt, unidentified
  source 1..228: mol_type = other RNA
  misc_feature 1..228: note = A18
tcaaccaaatatgtccaacgaaaggagcaatgccgggcctacatcgagcgacaaaccacaacaaccgaatccgacgatatcgagaagtcggaaactgattcggctgggcccacagccgaagggtgagggctaagcgccactcaccaaccccgcatgcgcaatatattgcgacttggctcgtcccacagcacaacatggcagaaagcccacgcgtgccgggatgggtcg

SEQ ID NO: 24 - RNA, 220 nt, unidentified
  source 1..220: mol_type = other RNA
  misc_feature 1..220: note = A19
tcaaccaaatatgtccaacgaaaggagcaatgccgggcctacatcgagcgacaaaccacaacaaccgaatccgacgatatcgagaagtcggaaactgattcggctgggcccacagccgaagggtgagggctaagcgccactcaccaaccccgcatgcgcaatatattgcgacttggctcgtcccacagcacaacatggcagaaagtgccgggatgggtcg

SEQ ID NO: 25 - RNA, 215 nt, unidentified
  source 1..215: mol_type = other RNA
  misc_feature 1..215: note = A20
tcaaccaaatatgtccaacgaaaggagcaatgccgggcctacatcgagcgacaaaccacaacaaccgaatccgacgatatcgagaagtcggaaactgattcggctgggcccacagccgaagggtgagggctaagcgccactcaccaaccccgcatgcgcaatatattgcgacttggctcgtcccacagcacaacatggcagaaagggatgggtcg

SEQ ID NO: 26 - RNA, 192 nt, unidentified
  source 1..192: mol_type = other RNA
  misc_feature 1..192: note = A1+A3
gcaatgccgggcctacatcgagcgacaaaccacaacaaccgaatccgacgatatcgagaagtcggaaactgattcggctgggcccacagccgaagggtgagggctaagcgccactcaccaaccccgcatgcttggctcgtcccacagcacaacatggcagaaaaacgagcccacgcgtgccgggatgggtcg

SEQ ID NO: 27 - RNA, 221 nt, unidentified
  source 1..221: mol_type = other RNA
  misc_feature 1..221: note = A1+A13
gtccaacgaaaggagcaatgccgggcctacatcgagcgacaaaccacaacaaccgaatccgacgatatcgagaagtcggaaactgattcggctgggcccacagccgaagggtgggggctaagcgccacccaccaaccccgcatgcgcaatatattgcgacttggctcgtcccacagcacaacatggcagaaaaacgagcccacgcgtgccgggatgggtcg

SEQ ID NO: 28 - RNA, 204 nt, unidentified
  source 1..204: mol_type = other RNA
  misc_feature 1..204: note = A3+A13
tcaaccaaatatgcaatgccgggcctacatcgagcgacaaaccacaacaaccgaatccgacgatatcgagaagtcggaaactgattcggctgggcccacagccgaagggtgggggctaagcgccacccaccaaccccgcatgcttggctcgtcccacagcacaacatggcagaaaaacgagcccacgcgtgccgggatgggtcg

SEQ ID NO: 29 - RNA, 234 nt, unidentified
  source 1..234: mol_type = other RNA
  misc_feature 1..234: note = A5+A6
tcaaccaaatatgtccaacgaaaggagcaacgccgggcctacatcgagcgacaaaccacaacaaccgaatccgacgatatcgagaagtcggaaactgattcggctgggcccacagccgaagggtgagggctaagcgccactcaccaaccccgcgttgcgcaatatattgcgacttggctcgtcccacagcacaacatggcagaaaaacgagcccacgcgtgccgggatgggtcg

SEQ ID NO: 30 - RNA, 233 nt, unidentified
  source 1..233: mol_type = other RNA
  misc_feature 1..233: note = A5+A13
tcaaccaaatatgtccaacgaaaggagcaacgccgggcctacatcgagcgacaaaccacaacaaccgaatccgacgatatcgagaagtcggaaactgattcggctgggcccacagccgaagggtgggggctaagcgccacccaccaaccccgcgtgcgcaatatattgcgacttggctcgtcccacagcacaacatggcagaaaaacgagcccacgcgtgccgggatgggtcg

SEQ ID NO: 31 - RNA, 224 nt, unidentified
  source 1..224: mol_type = other RNA
  misc_feature 1..224: note = A13+A17
tcaaccaaatatgtccaacgaaaggagcaatgccgggcctacatcgagcgacaaaccacaacaaccgaatccgacgatatcgagaagtcggaaactgattcggctgggcccacagccgaagggtgggggctaagcgccacccaccaaccccgcatgcgcaatatattgcgacttggctcgtcccacagcacgaaaaacgagcccacgcgtgccgggatgggtcg